European Patent Application EP 4 372 004 A1, published May 22, 2024. Title: CLDN18.2 binding molecules and use thereof. Applicant: SANYOU BIOPHARMACEUTICALS CO., LTD. Application WO. The sequence listing filed with the application follows.

SEQUENCE LISTING (12 sequences)

SEQ ID NO: 1 - protein, 10 aa, synthetic construct
  REGION 1..10: note = CDR1 of Nanobody Nb-NA3S-H1-T4
GSIFHIPVMG

SEQ ID NO: 2 - protein, 9 aa, synthetic construct
  REGION 1..9: note = CDR2 of Nanobody Nb-NA3S-H1-T4
GISRGGTTN

SEQ ID NO: 3 - protein, 12 aa, synthetic construct
  REGION 1..12: note = CDR3 of Nanobody Nb-NA3S-H1-T4 or of Nanobody Nb-NA3S-H1
LVVSGIGSTLEV

SEQ ID NO: 4 - protein, 120 aa, synthetic construct
  REGION 1..120: note = amino acid sequence of Nanobody Nb-NA3S-H1-T4
QVQLVESGGGLVQPGGSLRLSCAASGSIFHIPVMGWYRQAPGKQRELVAGISRGGTTNYGDSVKGRFTISRDNAKNTVYLQMNSLKPEDTAVYYCNVLVVSGIGSTLEVWGQGTLVTVSS

SEQ ID NO: 5 - protein, 120 aa, synthetic construct
  REGION 1..120: note = amino acid sequence of Nanobody Nb-NA3S-H1-T4-hVH6
QVQLVESGGGLVQPGGSLRLSCAASGSIFHIPVMGWYRQAPGKGLELVAGISRGGTTNYADSVKGRFTISRDNAKNTLYLQMNSLRAEDTAVYYCNVLVVSGIGSTLEVWGQGTLVTVSS

SEQ ID NO: 6 - protein, 232 aa, synthetic construct
  REGION 1..232: note = human IgG1 Fc region
EPKSCDKTHTCPPCPAPELLGGPSVFLFPPKPKDTLMISRTPEVTCVVVDVSHEDPEVKFNWYVDGVEVHNAKTKPREEQYNSTYRVVSVLTVLHQDWLNGKEYKCKVSNKALPAPIEKTISKAKGQPREPQVYTLPPSRDELTKNQVSLTCLVKGFYPSDIAVEWESNGQPENNYKTTPPVLDSDGSFFLYSKLTVDKSRWQQGNVFSCSVMHEALHNHYTQKSLSLSPGK

SEQ ID NO: 7 - protein, 352 aa, synthetic construct
  REGION 1..352: note = heavy chain antibody NA3SH1
QVQLVESGGGLVQPGGSLRLSCAASGSIFNIPVMGWYRQAPGKQRELVAGISTGGTTNYGDSVKGRFTISRDNAKNTVYLQMNSLKPEDTAVYYCNVLVVSGIGSTLEVWGQGTLVTVSSEPKSCDKTHTCPPCPAPELLGGPSVFLFPPKPKDTLMISRTPEVTCVVVDVSHEDPEVKFNWYVDGVEVHNAKTKPREEQYNSTYRVVSVLTVLHQDWLNGKEYKCKVSNKALPAPIEKTISKAKGQPREPQVYTLPPSRDELTKNQVSLTCLVKGFYPSDIAVEWESNGQPENNYKTTPPVLDSDGSFFLYSKLTVDKSRWQQGNVFSCSVMHEALHNHYTQKSLSLSPGK

SEQ ID NO: 8 - protein, 352 aa, synthetic construct
  REGION 1..352: note = heavy chain antibody NA3SH1-T4
QVQLVESGGGLVQPGGSLRLSCAASGSIFHIPVMGWYRQAPGKQRELVAGISRGGTTNYGDSVKGRFTISRDNAKNTVYLQMNSLKPEDTAVYYCNVLVVSGIGSTLEVWGQGTLVTVSSEPKSCDKTHTCPPCPAPELLGGPSVFLFPPKPKDTLMISRTPEVTCVVVDVSHEDPEVKFNWYVDGVEVHNAKTKPREEQYNSTYRVVSVLTVLHQDWLNGKEYKCKVSNKALPAPIEKTISKAKGQPREPQVYTLPPSRDELTKNQVSLTCLVKGFYPSDIAVEWESNGQPENNYKTTPPVLDSDGSFFLYSKLTVDKSRWQQGNVFSCSVMHEALHNHYTQKSLSLSPGK

SEQ ID NO: 9 - protein, 352 aa, synthetic construct
  REGION 1..352: note = heavy chain antibody NA3SH1-T4-hVH6
QVQLVESGGGLVQPGGSLRLSCAASGSIFHIPVMGWYRQAPGKGLELVAGISRGGTTNYADSVKGRFTISRDNAKNTLYLQMNSLRAEDTAVYYCNVLVVSGIGSTLEVWGQGTLVTVSSEPKSCDKTHTCPPCPAPELLGGPSVFLFPPKPKDTLMISRTPEVTCVVVDVSHEDPEVKFNWYVDGVEVHNAKTKPREEQYNSTYRVVSVLTVLHQDWLNGKEYKCKVSNKALPAPIEKTISKAKGQPREPQVYTLPPSRDELTKNQVSLTCLVKGFYPSDIAVEWESNGQPENNYKTTPPVLDSDGSFFLYSKLTVDKSRWQQGNVFSCSVMHEALHNHYTQKSLSLSPGK

SEQ ID NO: 10 - protein, 261 aa, synthetic construct
  REGION 1..261: note = hCLDN18.2
MAVTACQGLGFVVSLIGIAGIIAATCMDQWSTQDLYNNPVTAVFNYQGLWRSCVRESSGFTECRGYFTLLGLPAMLQAVRALMIVGIVLGAIGLLVSIFALKCIRIGSMEDSAKANMTLTSGIMFIVSGLCAIAGVSVFANMLVTNFWMSTANMYTGMGGMVQTVQTRYTFGAALFVGWVAGGLTLIGGVMMCIACRGLAPEETNYKAVSYHASGHSVAYKPGGFKASTGFGSNTKNKKIYDGGARTEDEVQSYPSKHDYV

SEQ ID NO: 11 - protein, 10 aa, synthetic construct
  REGION 1..10: note = CDR1 of Nanobody Nb-NA3S-H1
GSIFNIPVMG

SEQ ID NO: 12 - protein, 9 aa, synthetic construct
GISTGGTTN